European Patent Specification EP 3 999 520 B1, published August 30, 2023. Title: Complexe hybride htiARN / nanoparticule et son utilisation pour le traitement d'une maladie du systeme digestif. Applicant: Commissariat a l'energie atomique et aux energies alternatives. The sequence listing filed with the application follows.

SEQUENCE LISTING (9 sequences)

SEQ ID NO: 1 - DNA, 47 bp, Artificial Sequence
  premier brin d'ADN de l'hybride htiGFP
cgatctgagcgcgcttacggaacaggcaagctgaccctgaagttcat

SEQ ID NO: 2 - DNA, 47 bp, Artificial Sequence
  deuxieme brin d'ADN de l'hybride htiGFP
ccgtaagcgcgctcagatcgaacaggcaagctgaccctgaagttcat

SEQ ID NO: 3 - RNA, 22 nt, Homo sapiens
  modified_base (1)..(1): phosphorylated g
gaacuucagggucagcuugccg

SEQ ID NO: 4 - DNA, 22 bp, Artificial Sequence
  sequences nucleotidiques SC1 du premier brin d'ADN et SC2 du deuxieme brin d'ADN de l'hybride htiGFP
gcaagctgaccctgaagttcat

SEQ ID NO: 5 - DNA, 20 bp, Artificial Sequence
  sequence nucleotidique S1 du premier brin d'ADN de l'hybride htiGFP
cgatctgagcgcgcttacgg

SEQ ID NO: 6 - DNA, 20 bp, Artificial Sequence
  sequence nucleotidique S2 du deuxieme brin d'ADN de l'hybride htiGFP
ccgtaagcgcgctcagatcg

SEQ ID NO: 7 - RNA, 21 nt, Artificial Sequence
  ARN antisens non susceptible de moduler les mecanismes endogenes d'ARN interference de l'hybride htiCTRL
  modified_base (1)..(1): phosphorylated a
acgugacacguucggagaauu

SEQ ID NO: 8 - DNA, 46 bp, Artificial Sequence
  premier brin d'ADN de l'hybride htiCTRL
cgatctgagcgcgcttacggaacagttctccgaacgtgtcacgtat

SEQ ID NO: 9 - DNA, 46 bp, Artificial Sequence
  deuxieme brin d'ADN de l'hybride htiCTRL
ccgtaagcgcgctcagatcgaacagttctccgaacgtgtcacgtat